European Patent Specification EP 3 639 834 B1, published July 12, 2023. Title: Use of microbial communities for human and animal health. Applicant: Universiteit Gent. The sequence listing filed with the application follows.

SEQUENCE LISTING (7 sequences)

SEQ ID NO: 1 - DNA, 1485 bp, Roseburia hominis
gatcctggctcaggatgaacgctggcggcgtgcttaacacatgcaagtcgaacgaagcactttaattgatttcttcggaatgaagtttttgtgactgagtggcggacgggtgagtaacgcgtgggtaacctgcctcatacagggggataacagttggaaacgactgctaataccgcataagcgcacaggattgcatgatccagtgtgaaaaactccggtggtatgagatggacccgcgtctgattagccagttggcggggtaacggcccaccaaagcgacgatcagtagccgacctgagagggtgaccggccacattgggactgagacacggcccaaactcctacgggaggcagcagtggggaatattgcacaatgggggaaaccctgatgcagcgacgccgcgtgagcgaagaagtatttcggtatgtaaagctctatcagcagggaagaagaatgcggtacctgactaagaagcaccggctaaatacgtgccagcagccgcggtaatacgtatggtgcaagcgttatccggatttactgggtgtaaagggagcgcaggcggtacggcaagtctgatgtgaaatcccggggctcaaccccggtactgcattggaaactgtcggactagagtgtcggaggggtaagtggaattcctagtgtagcggtgaaatgcgtagatattaggaggaacaccagtggcgaaggcggcttactggacgattactgacgctgaggctcgaaagcgtggggagcaaacaggattagataccctggtagtccacgccgtaaacgatgaatactaggtgtcggggagcattgctcttcggtgccgcagcaaacgcaataagtattccacctggggagtacgttcgcaagaatgaaactcaaaggaattgacggggacccgcacaagcggtggagcatgtggtttaattcgaagcaacgcgaagaaccttaccaagtcttgacatcccactgacagagtatgtaatgtactttctcttcggagcagtggtgacaggtggtgcatggttgtcgtcagctcgtgtcgtgagatgttgggttaagtcccgcaacgagcgcaacccctattcttagtagccagcggttcggccgggcactctagggagactgccagggataacctggaggaaggtggggatgacgtcaaatcatcatgccccttatgacttgggctacacacgtgctacaatggcgtaaacaaagggaagcaatcccgcgagggggagcaaatctcaaaaataacgtctcagttcggactgtagtctgcaactcgactacacgaagctggaatcgctagtaatcgcgaatcagaatgtcgcggtgaatacgttcccgggtcttgtacacaccgcccgtcacaccatgggagttggtaatgcccgaagtcagtgacccaaccgcaaggagggagctgccgaaggcaggactgataactggggtgaagtcgtaacaagggtacg

SEQ ID NO: 2 - DNA, 1454 bp, Roseburia inulinivorans
ttgatcctggctcaggatgaacgctggcggcgtgcttaacacatgcaagtcgaacgaagcacttttacagatttcttcggaatgaagttttagtgactgagtggcggacgggtgagtaacgcgtgggtaacctgcctcacacagggggataacagttggaaacggctgctaataccgcataagcgcacagtaccgcatggtacagtgtgaaaaactccggtggtgtgagatggacccgcgtctgattagctagttggcagggcaacggcctaccaaggcgacgatcagtagccgacctgagagggtgaccggccacattgggactgagacacggcccaaactcctacgggaggcagcagtggggaatattgcacaatgggggaaaccctgatgcagcgacgccgcgtgagcgaagaagtatttcggtatgtaaagctctatcagcagggaagaagaaatgacggtacctgactaagaagcaccggctaaatacgtgccagcagccgcggtaatacgtatggtgcaagcgttatccggatttactgggtgtaaagggagcgcaggcggaaggctaagtctgatgtgaaagcccggggctcaaccccggtactgcattggaaactggtcatctagagtgtcggaggggtaagtggaattcctagtgtagcggtgaaatgcgtagatattaggaggaacaccagtggcgaaggcggcttactggacgataactgacgctgaggctcgaaagcgtggggagcaaacaggattagataccctggtagtccacgccgtaaacgatgaatactaggtgtcggaaagcacagcttttcggtgccgccgcaaacgcattaagtattccacctggggagtacgttcgcaagaatgaaactcaaaggaattgacggggacccgcacaagcggtggagcatgtggtttaattcgaagcaacgcgaagaaccttaccaagtcttgacatccttctgaccggacagtaatgtgtcctttccttcgggacagaagtgacaggtggtgcatggttgtcgtcagctcgtgtcgtgagatgttgggttaagtcccgcaacgagcgcaacccttatccccagtagccagcggttcggacgggcactctgaggagactgccagggataacctggaggaaggtggggatgacgtcaaatcatcatgccccttatgacttgggctacacacgtgctacaatggcgtaaacaaagggaagcgagaccgtgaggtggagcaaatcccaaaaataacgtctcagttcggactgtagtctgcaacccgactacacgaagctggaatcgctagtaatcgcagatcagaatgctgcggtgaatacgttcccgggtcttgtacacaccgcccgtcacaccatgggagttggaaatgcccgaagtcagtgacccaaccgcaaggagggagctgcgaaggcaggt

SEQ ID NO: 3 - DNA, 1433 bp, Akkermansia muciniphila
aacgaacgctggcggcgtggataagacatgcaagtcgaacgagagaattgctagcttgctaataattctctagtggcgcacgggtgagtaacacgtgagtaacctgcccccgagagcgggatagccctgggaaactgggattaataccgcatagtatcgaaagattaaagcagcaatgcgcttggggatgggctcgcggcctattagttagttggtgaggtaacggctcaccaaggcgatgacgggtagccggtctgagaggatgtccggccacactggaactgagacacggtccagacacctacgggtggcagcagtcgagaatcattcacaatgggggaaaccctgatggtgcgacgccgcgtgggggaatgaaggtcttcggattgtaaacccctgtcatgtgggagcaaattaaaaagatagtaccacaagaggaagagacggctaactctgtgccagcagccgcggtaatacagaggtctcaagcgttgttcggaatcactgggcgtaaagcgtgcgtaggctgtttcgtaagtcgtgtgtgaaaggcgcgggctcaacccgcggacggcacatgatactgcgagactagagtaatggagggggaaccggaattctcggtgtagcagtgaaatgcgtagatatcgagaggaacactcgtggcgaaggcgggttcctggacattaactgacgctgaggcacgaaggccaggggagcgaaagggattagatacccctgtagtcctggcagtaaacggtgcacgcttggtgtgcggggaatcgaccccctgcgtgccggagtaacgcgttaagcgtgccgcctggggagtacggtcgcaagattaaaactcaaagaaattgacggggacccgcacaagcggtggagtatgtggcttaattcgatgcaacgcgaagaaccttacctgggcttgacatgtaatgaacaacatgtgaaagcatgcgactcttcggaggcgttacacaggtgctgcatggccgtcgtcagctcgtgtcgtgagatgtttggttaagtccagcaacgagcgcaacccctgttgccagttaccagcacgtgaaggtggggactctggcgagactgcccagatcaactgggaggaaggtggggacgacgtcaggtcagtatggcccttatgcccagggctgcacacgtactacaatgcccagtacagagggggccgaagccgcgaggcggaggaaatcctaaaaactgggcccagttcggactgtaggctgcaacccgcctacacgaagccggaatcgctagtaatggcgcatcagctacggcgccgtgaatacgttcccgggtcttgtacacaccgcccgtcacatcatggaagctggtcgcacccgaagtatctgaagccaaccgcaaggaggcagggtcctaaggtgagactggtaactgggatg

SEQ ID NO: 4 - DNA, 1456 bp, Anaerostipes caccae
gcgcttaatacatgtcaagtcgaacgaagcatttaggattgaagttttcggatggatttcctatatgactgagtggcggacgggtgagtaacgcgtggggaacctgccctatacagggggataacagctggaaacggctgctaataccgcataagcgcacagaatcgcatgattcagtgtgaaaagccctggcagtataggatggtcccgcgtctgattagctggttggtgaggtaacggctcaccaaggcgacgatcagtagccggcttgagagagtgaacggccacattgggactgagacacggcccaaactcctacgggaggcagcagtggggaatattgcacaatgggggtaaaccctgatgcagcgacgccgcgtgagtgaagaagtatttcggtatgtaaagctctatcagcagggaagaaaacagacggtacctgactaagaagccccggctaactacgtgccagcagccgcggtaatacgtagggggcaagcgttatccggaattactgggtgtaaagggtgcgtaggtggcatggtaagtcagaagtgaaagcccggggcttaaccccgggactgcttttgaaactgtcatgctggagtgcaggagaggtaagcggaattcctagtgtagcggtgaaatgcgtagatattaggaggaacaccagtggcgaaggcggcttactggactgtcactgacactgatgcacgaaagcgtggggagcaaacaggattagataccctggtagtccacgccgtaaacgatgaatactaggtgtcggggccgtagaggcttcggtgccgcagcaaacgcagtaagtattccacctggggagtacgttcgcaagaatgaaactcaaaggaattgacggggacccgcacaagcggtggagcatgtggtttaattcgaagcaacgcgaagaaccttacctggtcttgacatcccaatgaccgaaccttaaccggttttttctttcgagacattggagacaggtggtgcatggttgtcgtcagctcgtgtcgtgagatgttgggttaagtcccgcaacgagcgcaacccctatctttagtagccagcatttaaggtgggcactctagagagactgccagggataacctggaggaaggtggggacgacgtcaaatcatcatgccccttatggccagggctacacacgtgctacaatggcgtaaacaaagggaagcgaagtcgtgaggcgaagcaaatcccagaaataacgtctcagttcggattgtagtctgcaactcgactacatgaagctggaatcgctagtaatcgtgaatcagaatgtcacggtgaatacgttcccgggtcttgtacacaccgcccgtcacaccatgggagtcagtaacgcccgaagtcagtgacccaaccgcaaggagggagctgccgaaggtgggaccgataactggggtgaagtcgtaacaagg

SEQ ID NO: 5 - DNA, 1466 bp, Faecalibacterium prausnitzii
gttgatcctggctcaggacgaacgctggcggcgcgcctaacacatgcaagtcgaacgagcgagagagagcttgctttctcgagcgagtggcgaacgggtgagtaacgcgtgaggaacctgcctcaaagagggggacaacagttggaaacgactgctaataccgcataagcccacagctcggcatcgagcagagggaaaaggagcaatccgctttgagatggcctcgcgtccgattagctagttggtgaggtaatggcccaccaaggcaacgatcggtagccggactgagaggttgaacggccacattgggactgagacacggcccagactcctacgggaggcagcagtggggaatattgcacaatgggggaaaccctgatgcagcgacgccgcgtggaggaagaaggtcttcggattgtaaactcctgttgttgaggaagataatgacggtactcaacaaggaagtgacggctaactacgtgccagcagccgcggtaaaacgtaggtcacaagcgttgtccggaattactgggtgtaaagggagcgcaggcgggaagacaagttggaagtgaaatctatgggctcaacccataaactgctttcaaaactgtttttcttgagtagtgcagaggtaggcggaattcccggtgtagcggtggaatgcgtagatatcgggaggaacaccagtggcgaaggcggcctactgggcaccaactgacgctgaggctcgaaagtgtgggtagcaaacaggattagataccctggtagtccacaccgtaaacgatgattactaggtgttggaggattgaccccttcagtgccgcagttaacacaataagtaatccacctggggagtacgaccgcaaggttgaaactcaaaggaattgacgggggcccgcacaagcagtggagtatgtggtttaattcgacgcaacgcgaagaaccttaccaagtcttgacatcctgcgacgatgctggaaacagtattttccttcgggacgcagagacaggtggtgcatggttgtcgtcagctcgtgtcgtgagatgttgggttaagtcccgcaacgagcgcaacccttactgtcagttactacgcaagaggactctggcaggactgccgttgacaaaacggaggaaggtggggatgacgtcaaatcatcatgccctttatgacttgggctacacacgtactacaatggcgttaaacaaagagaagcaagaccgcgaggtggagcaaaactcagaaacaacgtcccagttcggactgcaggctgcaactcgcctgcacgaagtcggaattgctagtaatcgtggatcagcatgccacggtgaatacgttcccgggccttgtacacaccgcccgtcacaccatgagagccggggggacccgaagtcggtagtctaaccgcaaggaggacgccgccgaaggtaaaactggtgattggggtgaagtcgtaacaaggtac

SEQ ID NO: 6 - DNA, 1586 bp, Lactobacillus plantarum
gggacatgctgcagtcgacgattagagtttgatcctggctcaggacgaacgctggcggcgtgcctaatacatgcaagtcgaacgaactctggtattgattggtgcttgcatcatgatttacatttgagtgagtggcgaactggtgagtaacacgtgggaaacctgcccagaagcgggggataacacctggaaacagatgctaataccgcataacaacttggaccgcatggtccgagtttgaaagatggcttcggctatcacttttggatggtcccgcggcgtattagctagatggtgaggtaacggcttaccatggcaatgatacgtagccgacctgagagggtaatcggccacattgggactgagacacggcccaaactcctacgggaggcagcagtagggaatcttccacaatggacgaaagtctgatggagcaacgccgcgtgagtgaagaagggtttcggctcgtaaaactctgttgttaaagaagaacatatctgagagtaactgttcaggtattgacggtatttaaccagaaagccacggctaactacgtgccagcagccgcggtaatacgtaggtggcaagcgttgtccggatttattgggcgtaaagcgagcgcaggcggttttttaagtctgatgtgaaagccttcggctcaaccgaagaagtgcatcggaaactgggaaacttgagtgcagaagaggacagtggaactccatgtgtagcggtgaaatgcgtagatatatggaagaacaccagtggcgaaggcggctgtctggtctgtaactgacgctgaggctcgaaagtatgggtagcaaacaggattagataccctggtagtccataccgtaaacgatgaatgctaagtgttggagggtttccgcccttcagtgctgcagctaacgcattaagcattccgcctggggagtacggccgcaaggctgaaactcaaaggaattgacgggggcccgcacaagcggtggagcatgtggtttaattcgaagctacgcgaagaaccttaccaggtcttgacatactatgcaaatctaagagattagacgttcccttcggggacatggatacaggtggtgcatggttgtcgtcagctcgtgtcgtgagatgttgggttaagtcccgcaacgagcgcaacccttattatcagttgccagcattaagttgggcactctggtgagactgccggtgacaaaccggaggaaggtggggatgacgtcaaatcatcatgccccttatgacctgggctacacacgtgctacaatggatggtacaacgagttgcgaactcgcgagagtaagctaatctcttaaagccattctcagttcggattgtaggctgcaactcgcctacatgaagtcggaatcgctagtaatcgcggatcagcatgccgcggtgaatacgttcccgggccttgtacacaccgcccgtcacaccatgagagtttgtaacacccaaagtcggtggggtaaccttttaggaaccagccgcctaaggtgggacagatgattagggtgaagtcgtaacaaggtaaccaatctctagaggtccccgggaccgagctgacgcaa

SEQ ID NO: 7 - DNA, 1482 bp, Butyricicoccus pullicaecorum
tagtttgatcctggctcaggatgaacgctggcggcgtgcctaacacatgcaagtcgaacggagttgtttgaggaaatccttcgggatggaatcttccaacttagtggcggacgggtgagtaacgcgtgagcaatctgcctttcagagggggataacagccggaaacggctgctaataccgcataatgcattgaattcgcatgtttttgatgccaaagattttatcgctgaaagatgagctcgcgtctgattagctagttggcggggtaacggcccaccaaggcgacgatcagtagccggactgagaggttgaacggccacattgggactgaggacacggcccagactcctaccgggaggcagcagtggggaatattgcgcaatgggggcaaccctgacgcagcaacgccgcgtgattgatgaaggtcttcggattgtaaaaatctttaatcagggacgaaacaaatgacggtacctgaagaataagctccggctaactacgtgccagcagccgcggtaatacgtagggagcaagcgttatccggatttactgggtgtaaagggcgtgtaggcgggcttgtaagttggaagtgaaatctcggggcttaaccccgaaactgctttcaaaactgcgagtcttgagtgatggagaggcaggcggaattcccagtgtagcggtgaaatgcgtagatattgggaggaacaccagtggcgaaggcggcctgctggacattaactgacgctgaggcgcgaaagcgtggggagcaaacaggattagataccctggtagtccacgccgtaaacgatggatactaggtgtgggaggtattgaccccttccgtgccggagttaacacaataagtatcccacctggggagtacggccgcaaggttgaaactcaaaggaattgacgggggcccgcacaagcagtggagtatgtggtttaattcgaagcaacgcgcaagaaccttaccaagtcttgacatcccgatgaccgctcyagagatagggcttttcttcggaacatcggtgacaggtggtgcatggttgtcgtcagctcgtgtcgtgagatgttgggttaagtcccgcaacgagcgcaacccttacgggttagttgctacgcaagagcactctagccggactgccgttgacaaaacggaggaaggtggggacgacgtcaaatcatcatgccccttatgacttgggctacacacgtactacaatggcagtcatacagagggaagcaaaaccgcgaggtggagcaaatccctaaaagctgtcccagttcagattgcaggctgcaactcgcctgcatgaagtcggaattgctagtaatcgcggatcagcatgccgcggtgaatacgttcccgggccttgtacacaccgcccgtcacaccatgagagccggtaatacccgaagtccgtagtctaaccgcaaggaggacgcggccgaaggtaggactggtaattgggacgaagtcgt